European Patent Application EP 4 393 516 A1, published July 3, 2024. Title: ANTIBODY FRAGMENT SPECIFIC TO C-KIT POSITIVE TUMORS. Applicant: TOKUSHIMA UNIVERSITY. Application EP. The sequence listing filed with the application follows.

SEQUENCE LISTING (23 sequences)

SEQ ID NO: 1 - DNA, 1383 bp, Mus musculus
  sig_peptide 1..57
  source 1..1383: mol_type = genomic DNA
  CDS 1..1383: protein_id = 2
atgggatggatctggatctttctcttcctcctgtcaggaactgcaggtgtccactctgaggtccagctgcagcagtctggacctgagctagtgaagactgggacttcagtgaagatatcctgcaaggcgtctggttactcattctctaattactacatgcactgggtcaagcagagccatggaaagagccttgagtggattggatatattagttgtttcaatggtgctactacctacaaccagaagttcaggggcaaggccacatttactgtagacacatcctccagcacaacctacatgcagttcaacagcctgacatctgaagactctgcggtctatttctgtgcaagacggacggctggagctatggactactggggtcaaggaacctcagtcaccgtctcctcagccaaaacgacacccccatctgtctatccactggcccctggatctgctgcccaaactaactccatggtgaccctgggatgcctggtcaagggctatttccctgagccagtgacagtgacctggaactctggatccctgtccagcggtgtgcacaccttcccagctgtcctgcagtctgacctctacactctgagcagctcagtgactgtcccctccagcacctggcccagcgagaccgtcacctgcaacgttgcccacccggccagcagcaccaaggtggacaagaaaattgtgcccagggattgtggttgtaagccttgcatatgtacagtcccagaagtatcatctgtcttcatcttccccccaaagcccaaggatgtgctcaccattactctgactcctaaggtcacgtgtgttgtggtagacatcagcaaggatgatcccgaggtccagttcagctggtttgtagatgatgtggaggtgcacacagctcagacgcaaccccgggaggagcagttcaacagcactttccgctcagtcagtgaacttcccatcatgcaccaggactggctcaatggcaaggagttcaaatgcagggtcaacagtgcagctttccctgcccccatcgagaaaaccatctccaaaaccaaaggcagaccgaaggctccacaggtgtacaccattccacctcccaaggagcagatggccaaggataaagtcagtctgacctgcatgataacagacttcttccctgaagacattactgtggagtggcagtggaatgggcagccagcggagaactacaagaacactcagcccatcatggacacagatggctcttacttcgtctacagcaagctcaatgtgcagaagagcaactgggaggcaggaaatactttcacctgctctgtgttacatgagggcctgcacaaccaccatactgagaagagcctctcccactctcctggtaaataa

SEQ ID NO: 2 - protein, 460 aa, Mus musculus
MGWIWIFLFLLSGTAGVHSEVQLQQSGPELVKTGTSVKISCKASGYSFSNYYMHWVKQSHGKSLEWIGYISCFNGATTYNQKFRGKATFTVDTSSSTTYMQFNSLTSEDSAVYFCARRTAGAMDYWGQGTSVTVSSAKTTPPSVYPLAPGSAAQTNSMVTLGCLVKGYFPEPVTVTWNSGSLSSGVHTFPAVLQSDLYTLSSSVTVPSSTWPSETVTCNVAHPASSTKVDKKIVPRDCGCKPCICTVPEVSSVFIFPPKPKDVLTITLTPKVTCVVVDISKDDPEVQFSWFVDDVEVHTAQTQPREEQFNSTFRSVSELPIMHQDWLNGKEFKCRVNSAAFPAPIEKTISKTKGRPKAPQVYTIPPPKEQMAKDKVSLTCMITDFFPEDITVEWQWNGQPAENYKNTQPIMDTDGSYFVYSKLNVQKSNWEAGNTFTCSVLHEGLHNHHTEKSLSHSPGK

SEQ ID NO: 3 - DNA, 720 bp, Mus musculus
  sig_peptide 1..60
  source 1..720: mol_type = genomic DNA
  CDS 1..720: protein_id = 4
atgaatttgcctgttcatctcttggtgcttctgttgttctggattcctgcttccagaggtgaagttgtggtgactcaaactccactctccctgcctgtcagctttggagatcaagtttctatctcttgcaggtctagtcagagtcttgcaaacagttatgggaacacctatttgtcttggtacctgcacaagcctggccagtctccacagctcctcatctatgggatttccaacagattttctggggtgccagacaggttcagtggcagtggttcagggacagagttcacactcgagatcagtacaataaagcctgaggacttgggaatgtattactgcttacaaggtacacatcagccgtacacgttcggaggggggaccaagctggaaataaaacgggctgatgctgcaccaactgtatccatcttcccaccatccagtgagcagttaacatctggaggtgcctcagtcgtgtgcttcttgaacaacttctaccccaaagacatcaatgtcaagtggaagattgatggcagtgaacgacaaaatggcgtcctgaacagttggactgatcaggacagcaaagacagcacctacagcatgagcagcaccctcacgttgaccaaggacgagtatgaacgacataacagctatacctgtgaggccactcacaagacatcaacttcacccattgtcaagagcttcaacaggaatgagtgttag

SEQ ID NO: 4 - protein, 239 aa, Mus musculus
MNLPVHLLVLLLFWIPASRGEVVVTQTPLSLPVSFGDQVSISCRSSQSLANSYGNTYLSWYLHKPGQSPQLLIYGISNRFSGVPDRFSGSGSGTEFTLEISTIKPEDLGMYYCLQGTHQPYTFGGGTKLEIKRADAAPTVSIFPPSSEQLTSGGASVVCFLNNFYPKDINVKWKIDGSERQNGVLNSWTDQDSKDSTYSMSSTLTLTKDEYERHNSYTCEATHKTSTSPIVKSFNRNEC

SEQ ID NO: 5 - DNA, 747 bp, Mus musculus
  sig_peptide 1..57
  source 1..747: mol_type = genomic DNA
  CDS 1..747: protein_id = 6
atgggatggatctggatctttctcttcctcctgtcaggaactgcaggtgtccactctgaggtccagctgcagcagtctggacctgagctagtgaagactgggacttcagtgaagatatcctgcaaggcgtctggttactcattctctaattactacatgcactgggtcaagcagagccatggaaagagccttgagtggattggatatattagttgtttcaatggtgctactacctacaaccagaagttcaggggcaaggccacatttactgtagacacatcctccagcacaacctacatgcagttcaacagcctgacatctgaagactctgcggtctatttctgtgcaagacggacggctggagctatggactactggggtcaaggaacctcagtcaccgtctcctcagccaaaacgacacccccatctgtctatccactggcccctggatctgctgcccaaactaactccatggtgaccctgggatgcctggtcaagggctatttccctgagccagtgacagtgacctggaactctggatccctgtccagcggtgtgcacaccttcccagctgtcctgcagtctgacctctacactctgagcagctcagtgactgtcccctccagcacctggcccagcgagaccgtcacctgcaacgttgcccacccggccagcagcaccaaggtggacaagaaaattgtgcccagggattgtggttgtaagccttgcatatgtacagtcccagaa

SEQ ID NO: 6 - protein, 249 aa, Mus musculus
MGWIWIFLFLLSGTAGVHSEVQLQQSGPELVKTGTSVKISCKASGYSFSNYYMHWVKQSHGKSLEWIGYISCFNGATTYNQKFRGKATFTVDTSSSTTYMQFNSLTSEDSAVYFCARRTAGAMDYWGQGTSVTVSSAKTTPPSVYPLAPGSAAQTNSMVTLGCLVKGYFPEPVTVTWNSGSLSSGVHTFPAVLQSDLYTLSSSVTVPSSTWPSETVTCNVAHPASSTKVDKKIVPRDCGCKPCICTVPE

SEQ ID NO: 7 - protein, 5 aa, Mus musculus
NYYMH

SEQ ID NO: 8 - protein, 17 aa, Mus musculus
YISCFNGATTYNQKFRG

SEQ ID NO: 9 - protein, 8 aa, Mus musculus
RTAGAMDY

SEQ ID NO: 10 - protein, 16 aa, Mus musculus
RSSQSLANSYGNTYLS

SEQ ID NO: 11 - protein, 7 aa, Mus musculus
GISNRFS

SEQ ID NO: 12 - protein, 9 aa, Mus musculus
LQGTHQPYT

SEQ ID NO: 13 - protein, 8 aa, Mus musculus
GYSFSNYY

SEQ ID NO: 14 - protein, 8 aa, Mus musculus
ISCFNGAT

SEQ ID NO: 15 - protein, 10 aa, Mus musculus
ARRTAGAMDY

SEQ ID NO: 16 - protein, 11 aa, Mus musculus
QSLANSYGNTY

SEQ ID NO: 17 - protein, 9 aa, Mus musculus
LQGTHQPYT

SEQ ID NO: 18 - DNA, 1401 bp, synthetic construct
  source 1..1401: mol_type = other DNA
  CDS 1..1401: protein_id = 19
atggactggacctggaggatcctctttttggtggcagcagccacaggtgcccactcccaggtccagcttgtgcagtctggggctgaggtgaagaagcctggggcctcagtgaaggtttcctgcaaggcttctggttactcattctctaattactacatgcactgggtgcgccaggcccccggacaaaggcttgagtggatgggatatattagttgtttcaatggtgctactacctacaaccagaagttcaggggcagagtcaccattaccagggacacatccgcgagcacagcctacatggagctgagcagcctgagatctgaagacacggctgtgtattactgtgcaagacggacggctggagctatggactactggggccagggaaccctggtcaccgtctcctcagctagcaccaagggcccatcggtcttccccctggcaccctcctccaagagcacctctgggggcacagcggccctgggctgcctggtcaaggactacttccccgaaccggtgacggtgtcgtggaactcaggcgccctgaccagcggcgtgcacaccttcccggctgtcctacagtcctcaggactctactccctcagcagcgtggtgaccgtgccctccagcagcttgggcacccagacctacatctgcaacgtgaatcacaagcccagcaacaccaaggtggacaagaaagttgagcccaaatcttgtgacaaaactcacacatgcccaccgtgcccagcacctgaactcctggggggaccgtcagtcttcctcttccccccaaaacccaaggacaccctcatgatctcccggacccctgaggtcacatgcgtggtggtggacgtgagccacgaagaccctgaggtcaagttcaactggtacgtggacggcgtggaggtgcataatgccaagacaaagccgcgggaggagcagtacaacagcacgtaccgtgtggtcagcgtcctcaccgtcctgcaccaggactggctgaatggcaaggagtacaagtgcaaggtctccaacaaagccctcccagcccccatcgagaaaaccatctccaaagccaaagggcagccccgagaaccacaggtgtacaccctgcccccatcccgggatgagctgaccaagaaccaggtcagcctgacctgcctggtcaaaggcttctatcccagcgacatcgccgtggagtgggagagcaatgggcagccggagaacaactacaagaccacgcctcccgtgctggactccgacggctccttcttcctctacagcaagctcaccgtggacaagagcaggtggcagcaggggaacgtcttctcatgctccgtgatgcatgaggctctgcacaaccactacacgcagaagagcctctccctgtctccgggtaaataa

SEQ ID NO: 19 - protein, 466 aa, synthetic construct
MDWTWRILFLVAAATGAHSQVQLVQSGAEVKKPGASVKVSCKASGYSFSNYYMHWVRQAPGQRLEWMGYISCFNGATTYNQKFRGRVTITRDTSASTAYMELSSLRSEDTAVYYCARRTAGAMDYWGQGTLVTVSSASTKGPSVFPLAPSSKSTSGGTAALGCLVKDYFPEPVTVSWNSGALTSGVHTFPAVLQSSGLYSLSSVVTVPSSSLGTQTYICNVNHKPSNTKVDKKVEPKSCDKTHTCPPCPAPELLGGPSVFLFPPKPKDTLMISRTPEVTCVVVDVSHEDPEVKFNWYVDGVEVHNAKTKPREEQYNSTYRVVSVLTVLHQDWLNGKEYKCKVSNKALPAPIEKTISKAKGQPREPQVYTLPPSRDELTKNQVSLTCLVKGFYPSDIAVEWESNGQPENNYKTTPPVLDSDGSFFLYSKLTVDKSRWQQGNVFSCSVMHEALHNHYTQKSLSLSPGK

SEQ ID NO: 20 - DNA, 720 bp, synthetic construct
  source 1..720: mol_type = other DNA
  CDS 1..720: protein_id = 21
atgaggctccctgctcagctcctggggctgctaatgctctggatccctggatccagtgcggatattgtgatgacccagactccactctctctgtccgtcacccctggacagccggcctccatctcctgcaggtctagtcagagtcttgcaaacagttatgggaacacctatttgtcttggtacctgcagaagccaggccagtctccacagctcctgatctatgggatttccaacagattttctggagtgccagataggttcagtggcagcgggtcagggacagatttcacactgaaaatcagccgggtggaggctgaggatgttggggtttattactgcttacaaggtacacatcagccgtacacgttcggcggagggaccaaggtggagatcaaacgaactgtggctgcaccatctgtcttcatcttcccgccatctgatgagcagttgaaatctggaactgcctctgttgtgtgcctgctgaataacttctatcccagagaggccaaagtacagtggaaggtggataacgccctccaatcgggtaactcccaggagagtgtcacagagcaggacagcaaggacagcacctacagcctcagcagcaccctgacgctgagcaaagcagactacgagaaacacaaagtctacgcctgcgaagtcacccatcagggcctgagcttgcccgtcacaaagagcttcaacaggggagagtgttag

SEQ ID NO: 21 - protein, 239 aa, synthetic construct
MRLPAQLLGLLMLWIPGSSADIVMTQTPLSLSVTPGQPASISCRSSQSLANSYGNTYLSWYLQKPGQSPQLLIYGISNRFSGVPDRFSGSGSGTDFTLKISRVEAEDVGVYYCLQGTHQPYTFGGGTKVEIKRTVAAPSVFIFPPSDEQLKSGTASVVCLLNNFYPREAKVQWKVDNALQSGNSQESVTEQDSKDSTYSLSSTLTLSKADYEKHKVYACEVTHQGLSLPVTKSFNRGEC

SEQ ID NO: 22 - DNA, 732 bp, synthetic construct
  source 1..732: mol_type = other DNA
  CDS 1..732: protein_id = 23
atggactggacctggaggatcctctttttggtggcagcagccacaggtgcccactcccaggtccagcttgtgcagtctggggctgaggtgaagaagcctggggcctcagtgaaggtttcctgcaaggcttctggttactcattctctaattactacatgcactgggtgcgccaggcccccggacaaaggcttgagtggatgggatatattagttgtttcaatggtgctactacctacaaccagaagttcaggggcagagtcaccattaccagggacacatccgcgagcacagcctacatggagctgagcagcctgagatctgaagacacggctgtgtattactgtgcaagacggacggctggagctatggactactggggccagggaaccctggtcaccgtctcctcagctagcaccaagggcccatcggtcttccccctggcaccctcctccaagagcacctctgggggcacagcggccctgggctgcctggtcaaggactacttccccgaaccggtgacggtgtcgtggaactcaggcgccctgaccagcggcgtgcacaccttcccggctgtcctacagtcctcaggactctactccctcagcagcgtggtgaccgtgccctccagcagcttgggcacccagacctacatctgcaacgtgaatcacaagcccagcaacaccaaggtggacaagaaagttgagcccaaatcttgtgacaaaactcactaa

SEQ ID NO: 23 - protein, 243 aa, synthetic construct
MDWTWRILFLVAAATGAHSQVQLVQSGAEVKKPGASVKVSCKASGYSFSNYYMHWVRQAPGQRLEWMGYISCFNGATTYNQKFRGRVTITRDTSASTAYMELSSLRSEDTAVYYCARRTAGAMDYWGQGTLVTVSSASTKGPSVFPLAPSSKSTSGGTAALGCLVKDYFPEPVTVSWNSGALTSGVHTFPAVLQSSGLYSLSSVVTVPSSSLGTQTYICNVNHKPSNTKVDKKVEPKSCDKTH